European Patent Application EP 4 635 954 A1, published October 22, 2025. Title: 一种诱导间质细胞向上皮细胞转化及重编程的诱导剂. Applicant: 武汉睿健医药科技有限公司. Application WO. The sequence listing filed with the application follows.

SEQUENCE LISTING (14 sequences)

SEQ ID NO: 1 - DNA, 20 bp, unidentified
  source 1..20: mol_type = unassigned DNA
ccatgcattcaaactgaggt

SEQ ID NO: 2 - DNA, 21 bp, unidentified
  source 1..21: mol_type = unassigned DNA
cctttgtgttcccaattcctt

SEQ ID NO: 3 - DNA, 22 bp, unidentified
  source 1..22: mol_type = unassigned DNA
acctcagctacaaacaggtgaa

SEQ ID NO: 4 - DNA, 20 bp, unidentified
  source 1..20: mol_type = unassigned DNA
aaaggctggggtaggtaggt

SEQ ID NO: 5 - DNA, 22 bp, unidentified
  source 1..22: mol_type = unassigned DNA
cagaagtcctacaaggtgtcca

SEQ ID NO: 6 - DNA, 21 bp, unidentified
  source 1..21: mol_type = unassigned DNA
ctctggttgaccgtaactgcg

SEQ ID NO: 7 - DNA, 22 bp, unidentified
  source 1..22: mol_type = unassigned DNA
tcgcaaatactgtggacaatgc

SEQ ID NO: 8 - DNA, 21 bp, unidentified
  source 1..21: mol_type = unassigned DNA
gcagtcgtgtgatattggtgt

SEQ ID NO: 9 - DNA, 21 bp, unidentified
  source 1..21: mol_type = other DNA
accaagtttgagacggaacag

SEQ ID NO: 10 - DNA, 21 bp, unidentified
  source 1..21: mol_type = unassigned DNA
ccctcagcgtactgatttcct

SEQ ID NO: 11 - DNA, 19 bp, unidentified
  source 1..19: mol_type = unassigned DNA
agaagatgcgctcgtcaaa

SEQ ID NO: 12 - DNA, 19 bp, unidentified
  source 1..19: mol_type = unassigned DNA
ggcttacggttcgtcttgt

SEQ ID NO: 13 - DNA, 22 bp, unidentified
  source 1..22: mol_type = unassigned DNA
ggccgaggactttgattgcaca

SEQ ID NO: 14 - DNA, 23 bp, unidentified
  source 1..23: mol_type = other DNA
gggcacgaaggctcatcattcaa